European Patent Application EP 4 751 713 A1, published June 3, 2026. Title: Composition for Improving Skin Condition Comprising Peptide Complex As Active Ingredient. Applicant: CAREGEN CO., LTD. The sequence listing filed with the application follows.

SEQUENCE LISTING (18 sequences)

SEQ ID NO: 1 - protein, 9 aa, synthetic construct
KGSATGWMA

SEQ ID NO: 2 - protein, 5 aa, synthetic construct
LKTRN

SEQ ID NO: 3 - DNA, 21 bp, synthetic construct
  source 1..21: mol_type = other DNA
aacatccaaccttcccaaacg

SEQ ID NO: 4 - DNA, 21 bp, synthetic construct
  source 1..21: mol_type = other DNA
gaccctaagcccccaattctc

SEQ ID NO: 5 - DNA, 20 bp, synthetic construct
  source 1..20: mol_type = other DNA
ttcgacacatgggataacga

SEQ ID NO: 6 - DNA, 20 bp, synthetic construct
  source 1..20: mol_type = other DNA
tctttcaacacgcaggacag

SEQ ID NO: 7 - DNA, 20 bp, synthetic construct
  source 1..20: mol_type = other DNA
aaagaggcactgccagaaaa

SEQ ID NO: 8 - DNA, 20 bp, synthetic construct
  source 1..20: mol_type = other DNA
atctgaggtgcccatgctac

SEQ ID NO: 9 - DNA, 20 bp, synthetic construct
  source 1..20: mol_type = other DNA
tgagtggtagccagcaaagc

SEQ ID NO: 10 - DNA, 20 bp, synthetic construct
  source 1..20: mol_type = other DNA
ctgcagtccaggttcaatgg

SEQ ID NO: 11 - DNA, 22 bp, synthetic construct
  source 1..22: mol_type = other DNA
ccacagaccttccaggagaatg

SEQ ID NO: 12 - DNA, 23 bp, synthetic construct
  source 1..23: mol_type = other DNA
gtgcagttcagtgatcgtacagg

SEQ ID NO: 13 - DNA, 20 bp, synthetic construct
  source 1..20: mol_type = other DNA
cacggccttccctacttcac

SEQ ID NO: 14 - DNA, 20 bp, synthetic construct
  source 1..20: mol_type = other DNA
agccactccttctgtgactc

SEQ ID NO: 15 - DNA, 20 bp, synthetic construct
  source 1..20: mol_type = other DNA
ggagccaaaagggtcatcat

SEQ ID NO: 16 - DNA, 20 bp, synthetic construct
  source 1..20: mol_type = other DNA
gtgatggcatggactgtggt

SEQ ID NO: 17 - DNA, 20 bp, synthetic construct
  source 1..20: mol_type = other DNA
ggtcccgtcgtctgtgatac

SEQ ID NO: 18 - DNA, 20 bp, synthetic construct
  source 1..20: mol_type = other DNA
tagcttttctggagagcgcc